European Patent Application EP 4 667 566 A9, published July 22, 2026. Title: 精氨酸脱亚胺酶突变体、共价二聚体及其偶联物和应用. Applicant: 重庆派金生物科技有限公司. The sequence listing filed with the application follows.

SEQUENCE LISTING (11 sequences)

SEQ ID NO: 1 - protein, 408 aa, synthetic construct
SVFDSKFNGIHVYSEIGELETVLVHEPGREIDYITPARLDELLFSAILESHDARKEHQSFVKIMKDRGINVVELTDLVAETYDLASKAAKEEFIETFLEETVPVLTEANKKAVRAFLLSKPTHEMVEFMMSGITKYELGVESENELIVDPMPNLYFTRDPFASVGNGVTIHFMRYIVRRRETLFARFVFRNHPKLVKTPWYYDPAMKMPIEGGDVFIYNNETLVVGVSERTDLDTITLLAKNIKANKEVEFKRIVAINVPKWTNLMHLDTWLTMLDKNKFLYSPIANDVFKFWDYDLVNGGAEPQPQLNGLPLDKLLASIINKEPVLIPIGGAGATEMEIARETNFDGTNYLAIKPGLVIGYDRNEKTNAALKAAGITVLPFHGNQLSLGMGNARCMSMPLSRKDVKW

SEQ ID NO: 2 - protein, 408 aa, synthetic construct
SVFDSKFNGIHVYSEIGELETVLVHEPGREIDYITPARLDELLFSCILESHDARKEHQSFVKIMKDRGINVVELTDLVAETYDLASKAAKEEFIETFLEETVPVLTEANKKAVRAFLLSKPTHEMVEFMMSGITKYELGVESENELIVDPMPNLYFTRDPFASVGNGVTIHFMRYIVRRRETLFARFVFRNHPKLVKTPWYYDPAMKMPIEGGDVFIYNNETLVVGVSERTDLDTITLLAKNIKANKEVEFKRIVAINVPKWTNLMHLDTWLTMLDKNKFLYSPIANDVFKFWDYDLVNGGAEPQPQLNGLPLDKLLASIINKEPVLIPIGGAGATEMEIARETNFDGTNYLAIKPGLVIGYDRNEKTNAALKAAGITVLPFHGNQLSLGMGNARCMSMPLSRKDVKW

SEQ ID NO: 3 - protein, 408 aa, synthetic construct
SVFDSKFNGIHVYSEIGELETVLVHEPGREIDYITPARLDELLFSAILESHDARKEHQSFVKIMKDRGINVVELTDLVAETYDLASKAAKEEFIETFLEETVPVLTEANKKAVRAFLLSKPTHEMVEFMMSGITKYELGVESENCLIVDPMPNLYFTRDPFASVGNGVTIHFMRYIVRRRETLFARFVFRNHPKLVKTPWYYDPAMKMPIEGGDVFIYNNETLVVGVSERTDLDTITLLAKNIKANKEVEFKRIVAINVPKWTNLMHLDTWLTMLDKNKFLYSPIANDVFKFWDYDLVNGGAEPQPQLNGLPLDKLLASIINKEPVLIPIGGAGATEMEIARETNFDGTNYLAIKPGLVIGYDRNEKTNAALKAAGITVLPFHGNQLSLGMGNARCMSMPLSRKDVKW

SEQ ID NO: 4 - protein, 408 aa, synthetic construct
SVFDSKFNGIHVYSEIGELETVLVHEPGREIDYITPARLDELLFSAILESHDARKEHQSFVKIMKDRGINVVELTDLVAETYDLASKAAKEEFIETFLEETVPVLTEANKKAVRAFLLSKPTHEMVEFMMSGITKYELGVESENELIVDPMPNLYFTRDPFASVGNGVTIHFMRYIVRRRETLFARFVFRNHPKLVKTPWYYDPAMKMPIEGGDVFIYNNETLVVGVSERTDLDTITLLAKNIKANKEVEFKRIVAINVPKWTNLMHLDTWLTMLDKNKFLYSPIANDVFKFWDYDLVNGGAEPQPQLNGLPLDKLLASIINKEPVLIPIGGAGATCMEIARETNFDGTNYLAIKPGLVIGYDRNEKTNAALKAAGITVLPFHGNQLSLGMGNARCMSMPLSRKDVKW

SEQ ID NO: 5 - DNA, 1224 bp, synthetic construct
  source 1..1224: mol_type = other DNA
agcgtgttcgacagcaaatttaacggtatccacgtttacagcgaaattggcgagctggaaaccgtgctggttcacgaaccgggtcgtgagatcgactatattaccccggcgcgtctggatgagctgctgttcagcgcgatcctggaaagccacgacgcgcgtaaggagcaccagagctttgtgaagatcatgaaagatcgtggcattaacgtggttgaactgaccgacctggttgcggagacctacgatctggcgagcaaggcggcgaaagaggaattcatcgaaacctttctggaggaaaccgtgccggttctgaccgaggcgaacaagaaagcggtgcgtgcgttcctgctgagcaaaccgacccacgaaatggttgagtttatgatgagcggtatcaccaagtacgaactgggcgtggagagcgaaaacgagctgattgttgacccgatgccgaacctgtatttcacccgtgatccgtttgcgagcgtgggtaacggcgttaccatccacttcatgcgttacattgtgcgtcgtcgtgaaaccctgtttgcgcgtttcgtgtttcgtaaccacccgaagctggttaaaaccccgtggtactatgacccggcgatgaaaatgccgatcgagggtggcgatgtgttcatttataacaacgaaaccctggtggttggtgttagcgagcgtaccgacctggataccatcaccctgctggcgaagaacattaaagcgaacaaggaagttgagttcaaacgtatcgtggcgattaacgttccgaagtggaccaacctgatgcacctggacacctggctgaccatgctggataagaacaaatttctgtacagcccgatcgcgaacgacgtgttcaaattttgggactatgatctggttaacggtggcgcggaaccgcagccgcaactgaacggtctgccgctggataaactgctggcgagcatcattaacaaggaaccggtgctgatcccgattggtggcgcgggtgcgaccgaaatggagatcgcgcgtgagaccaacttcgacggcaccaactacctggcgatcaagccgggtctggtgattggctatgatcgtaacgagaaaaccaacgcggcgctgaaggcggcgggtattaccgttctgccgtttcacggcaaccaactgagcctgggtatgggcaacgcgcgttgcatgagcatgccgctgagccgtaaagatgttaagtgg

SEQ ID NO: 6 - DNA, 1224 bp, synthetic construct
  source 1..1224: mol_type = other DNA
agcgtgttcgacagcaaatttaacggtatccacgtttacagcgaaattggcgagctggaaaccgtgctggttcacgaaccgggtcgtgagatcgactatattaccccggcgcgtctggatgagctgctgttcagctgcatcctggaaagccacgacgcgcgtaaggagcaccagagctttgtgaagatcatgaaagatcgtggcattaacgtggttgaactgaccgacctggttgcggagacctacgatctggcgagcaaggcggcgaaagaggaattcatcgaaacctttctggaggaaaccgtgccggttctgaccgaggcgaacaagaaagcggtgcgtgcgttcctgctgagcaaaccgacccacgaaatggttgagtttatgatgagcggtatcaccaagtacgaactgggcgtggagagcgaaaacgagctgattgttgacccgatgccgaacctgtatttcacccgtgatccgtttgcgagcgtgggtaacggcgttaccatccacttcatgcgttacattgtgcgtcgtcgtgaaaccctgtttgcgcgtttcgtgtttcgtaaccacccgaagctggttaaaaccccgtggtactatgacccggcgatgaaaatgccgatcgagggtggcgatgtgttcatttataacaacgaaaccctggtggttggtgttagcgagcgtaccgacctggataccatcaccctgctggcgaagaacattaaagcgaacaaggaagttgagttcaaacgtatcgtggcgattaacgttccgaagtggaccaacctgatgcacctggacacctggctgaccatgctggataagaacaaatttctgtacagcccgatcgcgaacgacgtgttcaaattttgggactatgatctggttaacggtggcgcggaaccgcagccgcaactgaacggtctgccgctggataaactgctggcgagcatcattaacaaggaaccggtgctgatcccgattggtggcgcgggtgcgaccgaaatggagatcgcgcgtgagaccaacttcgacggcaccaactacctggcgatcaagccgggtctggtgattggctatgatcgtaacgagaaaaccaacgcggcgctgaaggcggcgggtattaccgttctgccgtttcacggcaaccaactgagcctgggtatgggcaacgcgcgttgcatgagcatgccgctgagccgtaaagatgttaagtgg

SEQ ID NO: 7 - DNA, 1224 bp, synthetic construct
  source 1..1224: mol_type = other DNA
agcgtgttcgacagcaaatttaacggtatccacgtttacagcgaaattggcgagctggaaaccgtgctggttcacgaaccgggtcgtgagatcgactatattaccccggcgcgtctggatgagctgctgttcagcgcgatcctggaaagccacgacgcgcgtaaggagcaccagagctttgtgaagatcatgaaagatcgtggcattaacgtggttgaactgaccgacctggttgcggagacctacgatctggcgagcaaggcggcgaaagaggaattcatcgaaacctttctggaggaaaccgtgccggttctgaccgaggcgaacaagaaagcggtgcgtgcgttcctgctgagcaaaccgacccacgaaatggttgagtttatgatgagcggtatcaccaagtacgaactgggcgtggagagcgaaaactgcctgattgttgacccgatgccgaacctgtatttcacccgtgatccgtttgcgagcgtgggtaacggcgttaccatccacttcatgcgttacattgtgcgtcgtcgtgaaaccctgtttgcgcgtttcgtgtttcgtaaccacccgaagctggttaaaaccccgtggtactatgacccggcgatgaaaatgccgatcgagggtggcgatgtgttcatttataacaacgaaaccctggtggttggtgttagcgagcgtaccgacctggataccatcaccctgctggcgaagaacattaaagcgaacaaggaagttgagttcaaacgtatcgtggcgattaacgttccgaagtggaccaacctgatgcacctggacacctggctgaccatgctggataagaacaaatttctgtacagcccgatcgcgaacgacgtgttcaaattttgggactatgatctggttaacggtggcgcggaaccgcagccgcaactgaacggtctgccgctggataaactgctggcgagcatcattaacaaggaaccggtgctgatcccgattggtggcgcgggtgcgaccgaaatggagatcgcgcgtgagaccaacttcgacggcaccaactacctggcgatcaagccgggtctggtgattggctatgatcgtaacgagaaaaccaacgcggcgctgaaggcggcgggtattaccgttctgccgtttcacggcaaccaactgagcctgggtatgggcaacgcgcgttgcatgagcatgccgctgagccgtaaagatgttaagtgg

SEQ ID NO: 8 - DNA, 1224 bp, synthetic construct
  source 1..1224: mol_type = other DNA
agcgtgttcgacagcaaatttaacggtatccacgtttacagcgaaattggcgagctggaaaccgtgctggttcacgaaccgggtcgtgagatcgactatattaccccggcgcgtctggatgagctgctgttcagcgcgatcctggaaagccacgacgcgcgtaaggagcaccagagctttgtgaagatcatgaaagatcgtggcattaacgtggttgaactgaccgacctggttgcggagacctacgatctggcgagcaaggcggcgaaagaggaattcatcgaaacctttctggaggaaaccgtgccggttctgaccgaggcgaacaagaaagcggtgcgtgcgttcctgctgagcaaaccgacccacgaaatggttgagtttatgatgagcggtatcaccaagtacgaactgggcgtggagagcgaaaacgagctgattgttgacccgatgccgaacctgtatttcacccgtgatccgtttgcgagcgtgggtaacggcgttaccatccacttcatgcgttacattgtgcgtcgtcgtgaaaccctgtttgcgcgtttcgtgtttcgtaaccacccgaagctggttaaaaccccgtggtactatgacccggcgatgaaaatgccgatcgagggtggcgatgtgttcatttataacaacgaaaccctggtggttggtgttagcgagcgtaccgacctggataccatcaccctgctggcgaagaacattaaagcgaacaaggaagttgagttcaaacgtatcgtggcgattaacgttccgaagtggaccaacctgatgcacctggacacctggctgaccatgctggataagaacaaatttctgtacagcccgatcgcgaacgacgtgttcaaattttgggactatgatctggttaacggtggcgcggaaccgcagccgcaactgaacggtctgccgctggataaactgctggcgagcatcattaacaaggaaccggtgctgatcccgattggtggcgcgggtgcgacctgcatggagatcgcgcgtgagaccaacttcgacggcaccaactacctggcgatcaagccgggtctggtgattggctatgatcgtaacgagaaaaccaacgcggcgctgaaggcggcgggtattaccgttctgccgtttcacggcaaccaactgagcctgggtatgggcaacgcgcgttgcatgagcatgccgctgagccgtaaagatgttaagtgg

SEQ ID NO: 9 - protein, 392 aa, synthetic construct
IHVYSEIGELETVLVHEPGREIDYITPARLDELLFSAILESHDARKEHQSFVKQLKDNGINVVELTDLVAETFDLASKEEQEKLIEEFLEDSEPVLSEAHKTAVRKFLTSRKSTREMVEFMMAGITKYDLGIEADHELIVDPMPNLYFTRDPFASVGNGVTIHYMRYKVRQRETLFSRFVFSNHPKLVKTPWYYDPAMKMSIEGGDVFIYNNDTLVVGVSERTDLETITLLAKNIKANKEVEFKRIVAINVPKWTNLMHLDTWLTMLDKDKFLYSPIANDVFKFWDYDLVNGGAEPQPKENGLPLEGLLQSIINKKPVLIPIAGNNASHIDIERETHFDGTNYLAIKPGVVIGYARNEKTNAALAAAGIKVLPFHGNQLSLGMGNARCMSMP

SEQ ID NO: 10 - protein, 409 aa, synthetic construct
SVFDSKFKGIHVYSEIGELESVLVHEPGREIDYITPARLDELLFSAILESHDARKEHKQFVAELKANDINVVELIDLVAETYDLASQEAKDKLIEEFLEDSEPVLSEEHKVVVRNFLKAKKTSRELVEIMMAGITKYDLGIEADHELIVDPMPNLYFTRDPFASVGNGVTIHYMRYKVRQRETLFSRFVFSNHPKLINTPWYYDPSLKLSIEGGDVFIYNNDTLVVGVSERTDLQTVTLLAKNIVANKECEFKRIVAINVPKWTNLMHLDTWLTMLDKDKFLYSPIANDVFKFWDYDLVNGGAEPQPVENGLPLEGLLQSIINKKPVLIPIAGEGASQMEIERETHFDGTNYLAIRPGVVIGYSRNEKTNAALEAAGIKVLPFHGNQLSLGMGNARCMSMPLSRKDVKW

SEQ ID NO: 11 - protein, 408 aa, synthetic construct
SVFDSKFKGIHVYSEIGELETVLVHEPGKEIDYITPARLDELLFSAILESHDARKEHKEFVAELKKRGINVVELVDLIVETYDLASKEAKEKLLEEFLDDSAPVLSDEHRAAVKKFLQSQKSTRSLVEYMIAGITKHDLKIESDLELIVDPMPNLYFTRDPFASVGNGVTIHYMRYKVRQRETLFSRFVFSNHPKLVNTPWYYDPAEGLSIEGGDVFIYNNDTLVVGVSERTDLQTITLLAKNIKANKECEFKRIVAINVPKWTNLMHLDTWLTMLDKDKFLYSPIANDVFKFWDYDLVNGGDAPQPVDNGLPLEDLLKSIIGKKPTLIPIAGAGASQIDIERETHFDGTNYLAVAPGIVIGYARNEKTNAALEAAGITVLPFRGNQLSLGMGNARCMSMPLSRKDVK